European Patent Application EP 4 613 278 A1, published September 10, 2025. Title: 락토바실러스 델브루키 subsp. 락티스 균주의 신규 용도. Applicant: 주식회사 종근당바이오. The sequence listing filed with the application follows.

SEQUENCE LISTING (3 sequences)

SEQ ID NO: 1 - DNA, 1561 bp, Lactobacillus delbrueckii
  source 1..1561: mol_type = genomic DNA
attgagagtttgatcctggctcaggacgaacgctggcggcgtgcctaatacatgcaagtcgagcgagctgaattcaaagatcccttcggggtgatttgttggacgctagcggcggatgggtgagtaacacgtgggcaatctgccctaaagactgggataccacttggaaacaggtgctaataccggataacaacatgaatcgcatgattcaagtttgaaaggcggcgcaagctgtcactttaggatgagcccgcggcgcattagctagttggtggggtaaaggcctaccaaggcaatgatgcgtagccgagttgagagactgatcggccacattgggactgagacacggcccaaactcctacgggaggcagcagtagggaatcttccacaatggacgcaagtctgatggagcaacgccgcgtgagtgaagaaggtcttcggatcgtaaagctctgttgttggtgaagaaggatagaggcagtaactggtctttatttgacggtaatcaaccagaaagtcacggctaactacgtgccagcagccgcggtaatacgtaggtggcaagcgttgtccggatttattgggcgtaaagcgagcgcaggcggaatgataagtctgatgtgaaagcccacggctcaaccgtggaactgcatcggaaactgtcattcttgagtgcagaagaggagagtggaactccatgtgtagcggtggaatgcgtagatatatggaggaacaccagtggcgaaggcggctctctggtctgcaactgacgctgaggctcgaaagcatgggtagcgaacaggattagataccctggtagtccatgccgtaaacgatgagcgctaggtgttggggactttccggtcctcagtgccgcagcaaacgcattaagcgctccgcctggggagtacgaccgcaaggttgaaactcaaaggaattgacgggggcccgcacaagcggtggagcatgtggtttaattcgaagcaacgcgaagaaccttaccaggtcttgacatcctgcgctacacctagagataggtggttcccctcggggacgcagagacaggtggtgcatggctgtcgtcagctcgtgtcgtgagatgttgggttaagtcccgcaacgagcgcaacccttgtctttagttgccatcattaagttgggcactctaaagagactgccggtgacaaaccggaggaaggtggggatgacgtcaagtcatcatgccccttatgacctgggctacacacgtgctacaatgggcagtacaacgagaagcgaacccgcgagggtaagcggatctcttaaagctgctctcagttcggactgcaggctgcaactcgcctgcacgaagctggaatcgctagtaatcgcggatcagcacgccgcggtgaatacgttcccgggccttgtacacaccgcccgtcacaccatggaagtctgcaatgcccaaagtcggtgagataacctttataggagtcagccgcctaaggcagggcagatgactggggtgaagtcgtaacaaggtagccgtaggagaacctgcggctggatcacctccttt

SEQ ID NO: 2 - DNA, 17 bp, Lactobacillus delbrueckii
  source 1..17: mol_type = genomic DNA
cctacgggnggcwgcag

SEQ ID NO: 3 - DNA, 21 bp, Lactobacillus delbrueckii
  source 1..21: mol_type = genomic DNA
gactachvgggtatctaatcc